European Patent Specification EP 4 244 385 B1, published January 1, 2025. Title: LOOP MEDIATED ISOTHERMAL NUCLEIC ACID AMPLIFICATION (LAMP) USING LNA-MODIFIED PRIMERS AND A METAL-BASED COLORIMETRIC METHOD FOR DETECTING AN AMPLIFICATION PRODUCT. Applicant: MultiplexDX, s.r.o. The sequence listing filed with the application follows.

SEQUENCE LISTING (70 sequences)

SEQ ID NO: 1 - DNA, 16 bp, Artificial
  Human RPP30-F3
gttgctcaggctggag

SEQ ID NO: 2 - DNA, 20 bp, Artificial
  Human RPP30-B3
atcctaggagtttgagacca

SEQ ID NO: 3 - DNA, 43 bp, Artificial
  Human RPP30-FIP
ccgctgcttgagaggctgacttttattcagctcactgcaacct

SEQ ID NO: 4 - DNA, 48 bp, Artificial
  Human RPP30-BIP
tgcactaccacacctggctattaaacatttcaacatagtgagaccatg

SEQ ID NO: 5 - DNA, 17 bp, Artificial
  Human RPP30-LF
agcgggaggatcacttg

SEQ ID NO: 6 - DNA, 18 bp, Artificial
  Human RPP30-LB
ttttttcccttgtagaga

SEQ ID NO: 7 - DNA, 18 bp, Artificial
  SARS-CoV-2 N-F3
aacacaagctttcggcag

SEQ ID NO: 8 - DNA, 22 bp, Artificial
  SARS-CoV-2 N-B3
gaaatttggatctttgtcatcc

SEQ ID NO: 9 - DNA, 41 bp, Artificial
  SARS-CoV-2 N-FIP
tgcggccaatgtttgtaatcagccaaggaaattttggggac

SEQ ID NO: 10 - DNA, 39 bp, Artificial
  SARS-CoV-2 N-BIP
cgcattggcatggaagtcactttgatggcacctgtgtag

SEQ ID NO: 11 - DNA, 19 bp, Artificial
  SARS-CoV-2 N-LF
ttccttgtctgattagttc

SEQ ID NO: 12 - DNA, 18 bp, Artificial
  SARS-CoV-2 N-LB
ttcgggaacgtggttgac

SEQ ID NO: 13 - DNA, 17 bp, Artificial
  SARS-CoV-2 RdRP-F3
ctgtgatgccatgcgaa

SEQ ID NO: 14 - DNA, 21 bp, Artificial
  SARS-CoV-2 RdRP-B3
cggtcaaagagttttaacctc

SEQ ID NO: 15 - DNA, 50 bp, Artificial
  SARS-CoV-2 RdRP-FIP
cgtggtttgtatgaaatcaccgaaatctgttgtattgttggtgtactgac

SEQ ID NO: 16 - DNA, 45 bp, Artificial
  SARS-CoV-2 RdRP-BIP
gaccagggctttaactgcagagctttatcccacttaatgtaaggc

SEQ ID NO: 17 - DNA, 25 bp, Artificial
  SARS-CoV-2 RdRP-LF
agttaccattgagatcttgattatc

SEQ ID NO: 18 - DNA, 23 bp, Artificial
  SARS-CoV-2 RdRP-LB
cacatgttgacactgacttaaca

SEQ ID NO: 19 - DNA, 19 bp, Artificial
  Human RPP30-forward
agatttggacctgcgagcg

SEQ ID NO: 20 - DNA, 20 bp, Artificial
  Human RPP30-reverse
gagcggctgtctccacaagt

SEQ ID NO: 21 - DNA, 19 bp, Artificial
  SARS-CoV-2 E1-F3
cgtttcggaagagacaggt

SEQ ID NO: 22 - DNA, 19 bp, Artificial
  SARS-CoV-2 E1-LNA(F3)
  misc_feature (3)..(3): LNA-T
  misc_feature (5)..(5): LNA-T
cgntncggaagagacaggt

SEQ ID NO: 23 - DNA, 19 bp, Artificial
  SARS-CoV-2 E1-B3
gaccagaagatcaggaact

SEQ ID NO: 24 - DNA, 19 bp, Artificial
  SARS-CoV-2 E1-LNA(B3)
  misc_feature (2)..(2): LNA-A
  misc_feature (5)..(5): LNA-A
  misc_feature (7)..(7): LNA-A
gnccngnagatcaggaact

SEQ ID NO: 25 - DNA, 50 bp, Artificial
  SARS-CoV-2 E1-FIP
cgcagtaaggatggctagtgttttttatagcgtacttctttttcttgctt

SEQ ID NO: 26 - DNA, 48 bp, Artificial
  SARS-CoV-2 E1-LNA(FIP)
  misc_feature (4)..(4): LNA-A
  misc_feature (6)..(6): LNA-T
  misc_feature (27)..(27): LNA-A
  misc_feature (28)..(28): LNA-T
  misc_feature (33)..(33): LNA-T
cgcngnaaggatggctagtgttttttnnagcgnacttctttttcttgc

SEQ ID NO: 27 - DNA, 45 bp, Artificial
  SARS-CoV-2 E1-BIP
cttcgattgtgtgcgtactgctgtttcagatttttaacacgagag

SEQ ID NO: 28 - DNA, 45 bp, Artificial
  SARS-CoV-2 E1-LNA(BIP)
  misc_feature (3)..(3): LNA-T
  misc_feature (25)..(25): LNA-thymidine
  misc_feature (26)..(26): LNA-T
  misc_feature (30)..(30): LNA-A
  misc_feature (31)..(31): LNA-T
ctncgattgtgtgcgtactgctgtnncagnnttttaacacgagag

SEQ ID NO: 29 - DNA, 20 bp, Artificial
  SARS-CoV-2 E1-LF
actagcaagaataccacgaa

SEQ ID NO: 30 - DNA, 20 bp, Artificial
  SARS-CoV-2 E1-LNA(LF)
  misc_feature (3)..(3): LNA-T
  misc_feature (4)..(4): LNA-A
  misc_feature (7)..(7): LNA-A
acnngcnagataaccacgaa

SEQ ID NO: 31 - DNA, 21 bp, Artificial
  SARS-CoV-2 E1-LNA(LF)
cgtgagtcttgtaaaaccttc

SEQ ID NO: 32 - DNA, 21 bp, Artificial
  SARS-CoV-2 E1-LNA(LB)
  misc_feature (3)..(3): LNA-T
  misc_feature (5)..(5): LNA-A
cgngngtcttgtaaaaccttc

SEQ ID NO: 33 - DNA, 21 bp, Artificial
  SARS-CoV-2 E2-F3
tgtactcattcgtttcggaag

SEQ ID NO: 34 - DNA, 21 bp, Artificial
  SARS-CoV-2 E2-LNA(F3)
  misc_feature (3)..(3): LNA-T
  misc_feature (6)..(6): LNA-T
tgnacncattcgtttcggaag

SEQ ID NO: 35 - DNA, 23 bp, Artificial
  SARS-CoV-2 E2-B3
caggaactctagaagaattcaga

SEQ ID NO: 36 - DNA, 23 bp, Artificial
  SARS-CoV-2 E2-LNA(B3)
  misc_feature (2)..(2): LNA-A
  misc_feature (4)..(4): LNA-G
  misc_feature (6)..(6): LNA-A
cngnanctctagaagaattcaga

SEQ ID NO: 37 - DNA, 47 bp, Artificial
  SARS-CoV-2 E2-FIP
cgcagtaaggatggctagtgtattttgcgtacttctttttcttgctt

SEQ ID NO: 38 - DNA, 47 bp, Artificial
  SARS-CoV-2 E2-LNA(FIP)
  misc_feature (4)..(4): LNA-A
  misc_feature (6)..(6): LNA-T
  misc_feature (30)..(30): LNA-T
  misc_feature (31)..(31): LNA-A
cgcngnaaggatggctagtgtattttgcgnncttctttttcttgctt

SEQ ID NO: 39 - DNA, 49 bp, Artificial
  SARS-CoV-2 E2-BIP
cttcgattgtgtgcgtactgcatttcgagagtaaacgtaaaaagaaggt

SEQ ID NO: 40 - DNA, 49 bp, Artificial
  SARS-CoV-2 E2-LNA(BIP)
  misc_feature (2)..(2): LNA-T
  misc_feature (3)..(3): LNA-T
  misc_feature (28)..(28): LNA-A
cnncgattgtgtgcgtactgcatttcgngagtaaacgtaaaaagaaggt

SEQ ID NO: 41 - DNA, 20 bp, Artificial
  SARS-CoV-2 E2-LF
actagcaagaataccacgaa

SEQ ID NO: 42 - DNA, 19 bp, Artificial
  SARS-CoV-2 E2-LNA(LF)
  misc_feature (1)..(1): LNA-A
  misc_feature (3)..(3): LNA-T
  misc_feature (4)..(4): LNA-A
ncnngcaagaataccacga

SEQ ID NO: 43 - DNA, 21 bp, Artificial
  SARS-CoV-2 E2-LB
cgtgagtcttgtaaaaccttc

SEQ ID NO: 44 - DNA, 20 bp, Artificial
  SARS-CoV-2 E2-LNA(LB)
  misc_feature (1)..(1): LNA-T
  misc_feature (4)..(4): LNA-A
  misc_feature (6)..(6): LNA-T
ngcnanattgttaacgtgag

SEQ ID NO: 45 - DNA, 21 bp, Artificial
  SARS-CoV-2 E3-F3
tactcattcgtttcggaagag

SEQ ID NO: 46 - DNA, 21 bp, Artificial
  SARS-CoV-2 E3-LNA(F3) [1]
  misc_feature (1)..(1): LNA-T
  misc_feature (4)..(4): LNA-T
nacncattcgtttcggaagag

SEQ ID NO: 47 - DNA, 21 bp, Artificial
  SARS-CoV-2 E3-LNA(F3) [2]
  misc_feature (2)..(2): LNA-A
  misc_feature (6)..(6): LNA-A
tnctcnttcgtttcggaagag

SEQ ID NO: 48 - DNA, 23 bp, Artificial
  SARS-CoV-2 E3-B3
caggaactctagaagaattcaga

SEQ ID NO: 49 - DNA, 23 bp, Artificial
  SARS-CoV-2 E3-LNA(B3) [1]
  misc_feature (2)..(2): LNA-A
  misc_feature (4)..(4): LNA-G
  misc_feature (6)..(6): LNA-A
cngnanctctagaagaattcaga

SEQ ID NO: 50 - DNA, 23 bp, Artificial
  SARS-CoV-2 E3-LNA(B3) [2]
  misc_feature (2)..(2): LNA-A
  misc_feature (5)..(5): LNA-A
cnggnactctagaagaattcaga

SEQ ID NO: 51 - DNA, 48 bp, Artificial
  SARS-CoV-2 E3-FIP
gtaaggatggctagtgtaactagccaggtacgttaatagttaatagcg

SEQ ID NO: 52 - DNA, 43 bp, Artificial
  SARS-CoV-2 E3-BIP
gcttcgattgtgtgcgtactcgagagtaaacgtaaaaagaagg

SEQ ID NO: 53 - DNA, 22 bp, Artificial
  SARS-CoV-2 E3-LF
ccacgaaagcaagaaaaagaag

SEQ ID NO: 54 - DNA, 22 bp, Artificial
  SARS-CoV-2 E3-LB
gctgcaatattgttaacgtgag

SEQ ID NO: 55 - DNA, 17 bp, Artificial
  SARS-CoV-2 R1-F3
ctgtgatgccatgcgaa

SEQ ID NO: 56 - DNA, 17 bp, Artificial
  SARS-CoV-2 R1-LNA(F3)
  misc_feature (2)..(2): LNA-T
  misc_feature (4)..(4): LNA-T
cngngatgccatgcgaa

SEQ ID NO: 57 - DNA, 21 bp, Artificial
  SARS-CoV-2 R1-B3
cggtcaaagagttttaacctc

SEQ ID NO: 58 - DNA, 21 bp, Artificial
  SARS-CoV-2 R1-LNA(B3)
  misc_feature (2)..(2): LNA-G
  misc_feature (4)..(4): LNA-T
  misc_feature (7)..(7): LNA-A
cngncanagagttttaacctc

SEQ ID NO: 59 - DNA, 50 bp, Artificial; identical to SEQ ID NO: 15
  SARS-CoV-2 R1-FIP

SEQ ID NO: 60 - DNA, 45 bp, Artificial; identical to SEQ ID NO: 16
  SARS-CoV-2 R1-BIP

SEQ ID NO: 61 - DNA, 25 bp, Artificial
  SARS-CoV-2 R1-LF
agttaccattgagatcttgattatc

SEQ ID NO: 62 - DNA, 23 bp, Artificial
  SARS-CoV-2 R1-LB
cacatgttgacactgacttaaca

SEQ ID NO: 63 - DNA, 18 bp, Artificial
  SARS-CoV-2 N1-F3
aacacaagctttcggcag

SEQ ID NO: 64 - DNA, 18 bp, Artificial
  SARS-CoV-2 N1-LNA(F3)
  misc_feature (2)..(2): LNA-A
  misc_feature (4)..(4): LNA-A
ancncaagctttcggcag

SEQ ID NO: 65 - DNA, 22 bp, Artificial
  SARS-CoV-2 N1-B3
gaaatttggatctttgtcatcc

SEQ ID NO: 66 - DNA, 22 bp, Artificial
  SARS-CoV-2 N1-LNA(B3)
  misc_feature (2)..(2): LNA-A
  misc_feature (3)..(3): LNA-A
  misc_feature (7)..(7): LNA-T
gnnattnggatctttgtcatcc

SEQ ID NO: 67 - DNA, 41 bp, Artificial; identical to SEQ ID NO: 9
  SARS-CoV-2 N1-FIP

SEQ ID NO: 68 - DNA, 39 bp, Artificial; identical to SEQ ID NO: 10
  SARS-CoV-2 N1-BIP

SEQ ID NO: 69 - DNA, 19 bp, Artificial
  SARS-CoV-2 N1-LF
ttccttgtctgattagttc

SEQ ID NO: 70 - DNA, 18 bp, Artificial
  SARS-CoV-2 N1-LB
accttcgggaacgtggtt